European Patent Specification EP 3 957 753 B1, published August 21, 2024. Title: Polymerase Chain Reaction Primers and Probes for Mycobacterium Tuberculosis. Applicant: Rutgers, the State University of New Jersey. The sequence listing filed with the application follows.

SEQUENCE LISTING (73 sequences)

SEQ ID NO: 1 - DNA, 19 bp, Artificial Sequence
  synthesized oligo
ccggtcggttgccgagacc

SEQ ID NO: 2 - DNA, 22 bp, Artificial Sequence
  synthesized oligo
cggtcggttgccgagaccatgg

SEQ ID NO: 3 - DNA, 22 bp, Artificial Sequence
  synthesized oligo
gtcggttgccgagaccatgggc

SEQ ID NO: 4 - DNA, 21 bp, Artificial Sequence
  synthesized oligo
agcgggtagcgcagcgaccag

SEQ ID NO: 5 - DNA, 22 bp, Artificial Sequence
  synthesized oligo
cgggtagcgcagcgaccagggc

SEQ ID NO: 6 - DNA, 23 bp, Artificial Sequence
  synthesized oligo
ccagcgggtagcgcagcgaccag

SEQ ID NO: 7 - DNA, 20 bp, Artificial Sequence
  synthesized oligo
gctggagcagatgggcttgg

SEQ ID NO: 8 - DNA, 22 bp, Artificial Sequence
  synthesized oligo
ccgctggagcagatgggcttgg

SEQ ID NO: 9 - DNA, 25 bp, Artificial Sequence
  synthesized oligo
ggctggaagagctcgtatggcaccg

SEQ ID NO: 10 - DNA, 26 bp, Artificial Sequence
  synthesized oligo
gtcccatttcgtcggggtgttcgtcc

SEQ ID NO: 11 - DNA, 27 bp, Artificial Sequence
  synthesized oligo
ccatttcgtcggggtgttcgtccatac

SEQ ID NO: 12 - DNA, 23 bp, Artificial Sequence
  synthesized oligo
cgtcgcggacctccagcccggca

SEQ ID NO: 13 - DNA, 21 bp, Artificial Sequence
  synthesized oligo
tcacgtgacagaccgccgggc

SEQ ID NO: 14 - DNA, 23 bp, Artificial Sequence
  synthesized oligo
gctcacgtgacagaccgccgggc

SEQ ID NO: 15 - DNA, 28 bp, Artificial Sequence
  synthesized oligo
gctagtaatcgcagatcagcaacgctgc

SEQ ID NO: 16 - DNA, 23 bp, Artificial Sequence
  synthesized oligo
cctcccgagggttaggccactgg

SEQ ID NO: 17 - DNA, 20 bp, Artificial Sequence
  synthesized oligo
ggttaggccactggcttcgg

SEQ ID NO: 18 - DNA, 23 bp, Artificial Sequence
  synthesized oligo
cacagggtcacagtcacagaatc

SEQ ID NO: 19 - DNA, 23 bp, Artificial Sequence
  synthesized oligo
cgtcctcggtcgggctacacagg

SEQ ID NO: 20 - DNA, 25 bp, Artificial Sequence
  synthesized oligo
cggtcgggctacacagggtcacagt

SEQ ID NO: 21 - DNA, 23 bp, Artificial Sequence
  synthesized oligo
cacagggtcacagtcacagaatc

SEQ ID NO: 22 - DNA, 25 bp, Artificial Sequence
  synthesized oligo
gcatcgcgtgatcctttgccagaca

SEQ ID NO: 23 - DNA, 24 bp, Artificial Sequence
  synthesized oligo
ctcgccggtgccagcggatatgtc

SEQ ID NO: 24 - DNA, 24 bp, Artificial Sequence
  synthesized oligo
cgaccgtccagcgcccacatcttt

SEQ ID NO: 25 - DNA, 21 bp, Artificial Sequence
  synthesized oligo
ccgcgagggccccgatggttt

SEQ ID NO: 26 - DNA, 23 bp, Artificial Sequence
  synthesized oligo
ggctgggctcccggttgatgtgg

SEQ ID NO: 27 - DNA, 24 bp, Artificial Sequence
  synthesized oligo
ggctcccggttgatgtggtcgtag

SEQ ID NO: 28 - DNA, 22 bp, Artificial Sequence
  synthesized oligo
tggggcgatcggcacacccagc

SEQ ID NO: 29 - DNA, 24 bp, Artificial Sequence
  synthesized oligo
atcggtggattgcccggcaagctg

SEQ ID NO: 30 - DNA, 23 bp, Artificial Sequence
  synthesized oligo
cgttccacggatccgcgcaagtc

SEQ ID NO: 31 - DNA, 22 bp, Artificial Sequence
  synthesized oligo
gctggccgattgccgttccacg

SEQ ID NO: 32 - DNA, 23 bp, Artificial Sequence
  synthesized oligo
gatcatcaatgtggagaaagcgc

SEQ ID NO: 33 - DNA, 25 bp, Artificial Sequence
  synthesized oligo
ctggaacatcgaatcgcgaccgctt

SEQ ID NO: 34 - DNA, 22 bp, Artificial Sequence
  synthesized oligo
atcgcgaccgctttttgcagaa

SEQ ID NO: 35 - DNA, 21 bp, Artificial Sequence
  synthesized oligo
ctgaccgacgccgtggtgata

SEQ ID NO: 36 - DNA, 27 bp, Artificial Sequence
  synthesized oligo
ggaaatagttggacatgtagccggcgt

SEQ ID NO: 37 - DNA, 25 bp, Artificial Sequence
  synthesized oligo
cgattcgatgttccaggcgatactt

SEQ ID NO: 38 - DNA, 25 bp, Artificial Sequence
  synthesized oligo
gcgcggcaagatcatcaatgtggag

SEQ ID NO: 39 - DNA, 23 bp, Artificial Sequence
  synthesized oligo
gatcatcaatgtggagaaagcgc

SEQ ID NO: 40 - DNA, 22 bp, Artificial Sequence
  synthesized oligo
gtggatcccggtgcccagcgcc

SEQ ID NO: 41 - DNA, 22 bp, Artificial Sequence
  synthesized oligo
ggtgcccagcgccgtgatgatc

SEQ ID NO: 42 - DNA, 28 bp, Artificial Sequence
  synthesized oligo
cgttacgctcgtggacataccgatttcg

SEQ ID NO: 43 - DNA, 28 bp, Artificial Sequence
  synthesized oligo
ttacgctcgtggacataccgatttcggc

SEQ ID NO: 44 - DNA, 24 bp, Artificial Sequence
  synthesized oligo
ggactgaacgggatacgaatgggg

SEQ ID NO: 45 - DNA, 24 bp, Artificial Sequence
  synthesized oligo
gtttggccccttcagtggctgtgg

SEQ ID NO: 46 - DNA, 24 bp, Artificial Sequence
  synthesized oligo
cagcccgacgccgaatcagttgtt

SEQ ID NO: 47 - DNA, 21 bp, Artificial Sequence
  synthesized oligo
ggtgcgggcggtgtcgaggtg

SEQ ID NO: 48 - DNA, 21 bp, Artificial Sequence
  synthesized oligo
gccaccgcggggagtttgtcg

SEQ ID NO: 49 - DNA, 24 bp, Artificial Sequence
  synthesized oligo
atcaacatccggccggtggtcgcc

SEQ ID NO: 50 - DNA, 24 bp, Artificial Sequence
  synthesized oligo
agctccagcccggcacgctcacgt

SEQ ID NO: 51 - DNA, 28 bp, Artificial Sequence
  synthesized oligo
gctagtaatcgcagatcagcaacgctgc

SEQ ID NO: 52 - DNA, 21 bp, Artificial Sequence
  synthesized oligo
cctcccgagggttaggccact

SEQ ID NO: 53 - DNA, 24 bp, Artificial Sequence
  synthesized oligo
gcatcgcgtgatcctttgccagac

SEQ ID NO: 54 - DNA, 40 bp, Artificial Sequence
  synthesized oligo
cctgcgcgcaccagggtgccctagatcgacgcgtcgcagg

SEQ ID NO: 55 - DNA, 38 bp, Artificial Sequence
  synthesized oligo
ccaggggtgucgtagatcgacgcgtcgccgcgccctgg

SEQ ID NO: 56 - DNA, 38 bp, Artificial Sequence
  synthesized oligo
ccggcgacatcaatggtgctggtgatcgcgtccgccgg

SEQ ID NO: 57 - DNA, 43 bp, Artificial Sequence
  synthesized oligo
cgcggccgacagttggcgcttgtgggttaaccccgacgccgcg

SEQ ID NO: 58 - DNA, 41 bp, Artificial Sequence
  synthesized oligo
cgcgcgccgggccccagcaccaacagtcggagcttcgcgcg

SEQ ID NO: 59 - DNA, 35 bp, Artificial Sequence
  synthesized oligo
cacgaccgcccgtcacgtcatgaaagtcggtcgtg

SEQ ID NO: 60 - DNA, 39 bp, Artificial Sequence
  synthesized oligo
agcggtcgtaatattcacgtgcacctggccgcggccgct

SEQ ID NO: 61 - DNA, 38 bp, Artificial Sequence
  synthesized oligo
ctcgcggcatatgccacagtcggattctctgacgcgag

SEQ ID NO: 62 - DNA, 40 bp, Artificial Sequence
  synthesized oligo
caggcggtcgtaatattcacgtgcacctggccgccgcctg

SEQ ID NO: 63 - DNA, 38 bp, Artificial Sequence
  synthesized oligo
cgagcgtatgtagtagaaggtgactcggccggcgctcg

SEQ ID NO: 64 - DNA, 43 bp, Artificial Sequence
  synthesized oligo
acctgccgcggcgagacgataggutgtaggggtgacggcaggt

SEQ ID NO: 65 - DNA, 53 bp, Artificial Sequence
  synthesized oligo
ccgagctgatcguctgaacttcggcgtuctttagcacccggtugatagctcgg

SEQ ID NO: 66 - DNA, 38 bp, Artificial Sequence
  synthesized oligo
caccggcgactcgggccacgtccaggatgtagccggtg

SEQ ID NO: 67 - DNA, 34 bp, Artificial Sequence
  synthesized oligo
cgcgcaccaatatgatcgggtactcgactgcgcg

SEQ ID NO: 68 - DNA, 36 bp, Artificial Sequence
  synthesized oligo
tcggccatcaagggaatggagttggcgcgcggccga

SEQ ID NO: 69 - DNA, 39 bp, Artificial Sequence
  synthesized oligo
ccgcgtgggtgtcgagtcgatctgcacacagctacgcgg

SEQ ID NO: 70 - DNA, 20 bp, Artificial Sequence
  synthesized oligo
aaacgcgcaggtcagaaaat

SEQ ID NO: 71 - DNA, 20 bp, Artificial Sequence
  synthesized oligo
cagtgtcttggctacctcga

SEQ ID NO: 72 - DNA, 19 bp, Artificial Sequence
  synthesized oligo
gtcggtactgacagtcccc

SEQ ID NO: 73 - DNA, 19 bp, Artificial Sequence
  synthesized oligo
atgcaacagcatccttgcg